European Patent Specification EP 3 518 947 B1, published July 5, 2023. Title: OPTIMIZED ONCOLYTIC VIRUSES AND USES THEREOF. Applicant: SATOR Therapeutics LLC. The sequence listing filed with the application follows.

SEQUENCE LISTING (2 sequences)

SEQ ID NO: 1 - DNA, 6630 bp, Poliovirus Sabin strain Type 1
atgggtgctcaggtttcatcacagaaagtgggcgcacatgaaaactcaaatagagcgtatggtggttctaccattaattacaccaccattaattattatagagattcagctagtaacgcggcttcgaaacaggacttctctcaagacccttccaagttcaccgagcccatcaaggatgtcctgataaaaacatccccaatgctaaactcgccaaacatagaggcttgcgggtatagcgatagagtactgcaattaacactgggaaactccactataaccacacaggaggcggctaattcagtagtcgcttatgggcgttggcctgaatatctgagggacagcgaagccaatccagtggaccagccgacagaaccagacgtcgctgcatgcaggttttatacgctagacaccgtgtcttggacgaaagagtcgcgagggtggtggtggaagttgcctgatgcactgcgggacatgggactctttggccaaaatatgtactaccactacctaggtaggtccgggtacaccgtgcatgtacagtgtaacgcctccaaattccaccagggggcactaggggtattcgccgtaccagagatgtgtctggccggggatagcaacaccactaccatgcacaccagctatcaaaatgccaatcctggcgagaaaggaggcactttcacgggtacgttcactcctgacgacaaccagacatcacctgcccgtaggttctgcccggtggattacctctttggaaatggcacgttattggggaatgcctttgtgttcccgcaccagataataaacctacggaccaacaactgtgctacactggtactcccttacgtgaactccctctcgatagatagtatggtaaagcacaataattggggaattgcaatattaccattggccccattaaattttgctagtgagtcctccccagagattccaatcaccttgaccatagcccctatgtgctgtgagttcaatggattaagaaacattaccctgccacgcttacagggcctgccggtcatgaacacccctggtagcaatcaatatcttactgcagacaacttccagtcaccgtgtgcgctgcctgaatttgatgtgaccccacctattgacatacccggtgaagttaagaacatgatggaattggcagaaatcgacaccatgattccctttgacttaagtgcaaaaaaaaagaacaccatggaaatgtatagggttcggttaagtgacaaaccacatacagacgatcccatactctgcctgtcactctctccagcttcagatcctaggttgtcacatactatgcttggagaaatcctaaattactacacacactgggcaggatccctgaagttcacgtttctgttctgtggatccatgatggcaactggcaaactgttggtgtcatacgcgcctcctggagccgacccaccaaagaagcgtaaggaggcgatgttgggaacacatgtgatctgggacataggactgcagtcctcatgtactatggtagtgccatggattagcaacaccacgtatcggcaaaccatagatgatagtttcaccgaaggcggatacatcagcgtcttctaccaaaccagaatagtcgtccctctttcgacacccagagagatggacatccttggttttgtgtcagcgtgtaatgacttcagcgtgcgcttgatgcgagataccacacatatagagcaaaaagcgctagcacaggggttaggtcagatgcttgaaagcatgattgacaacacagtccgtgaaacggtgggggcggcaacgtctagagacgctctcccaaacactgaagccagtggaccagcacactccaaggaaattccggcactcaccgcagtggaaactggggccacaaatccactagtcccttctgatacagtgcaaaccagacatgttgtacaacataggtcaaggtcagagtctagcatagagtctttcttcgcgcggggtgcatgcgtggccattataaccgtggataactcagcttccaccaagaataaggataagctatttacagtgtggaagatcacttataaagatactgtccagttacggaggaaattggagttcttcacctattctagatttgatatggaatttacctttgtggttactgcaaatttcactgagactaacaatgggcatgccttaaatcaagtgtaccaaattatgtacgtaccaccaggcgctccagtgcccgagaaatgggacgactacacatggcaaacctcatcaaatccatcaatcttttacacctacggaacagctccagcccggatctcggtaccgtatgttggtatttcgaacgcctattcacacttttacgacggtttttccaaagtaccactgaaggaccagtcggcagcactaggtgactccctctatggtgcagcatctctaaatgacttcggtattttggctgttagagtagtcaatgatcacaacccgaccaaggtcacctccaaaatcagagtgtatctaaaacccaaacacatcagagtctggtgcccgcgtccaccgagggcagtggcgtactacggccctggagtggattacaaggatggtacgcttacacccctctccaccaaggatctgaccacatatggattcggacaccaaaacaaagcggtgtacactgcaggttacaaaatttgcaactaccatttggccactcaggaagatttgcaaaacgcagtgaacgtcatgtggaatagagacctcttagtcacagaatcaagagcccagggcaccgattcaatcgcaaggtgcaattgcaacgcaggggtgtactactgcgagtctagaaggaaatactacccagtatccttcgttggcccaacgttccagtacatggaggctaataactattacccagctaggtaccagtcccatatgctcattggccatggattcgcatctccaggggattgtggtggcatactcagatgtcaccacggggtgatagggatcattactgctggtggagaagggttggttgcatttacagacattagagacttgtatgcctacgaagaagaagccatggaacaaggcatcaccaattacatagagtcacttggggccgcatttggaagtggatttactcagcagattggagacaaaataacagagttgactaatatggtgaccagtaccatcactgaaaagctacttaagaacttgatcaagatcatatcctcactagttattataactaggaattatgaagacaccacaacagtgctcgctaccctggcccttcttgggtgtgatgcttcaccatggcagtggcttagaaagaaagcatgcgatgttctggagataccttatgtcaccaagcaaggtgacagttggttgaagaagtttactgaagcatgcaacgcagctaagggactggagtgggtgtcaaacaaaatctcaaaattcattgattggctcaaggagaaaattatcccacaagctagagataagttggaatttgtaacaaaacttagacaactagaaatgctggaaaaccaaatctcaactatacaccaatcatgccctagtcaggaacaccaggaaattctattcaataatgtcagatggttatccatccagtctaagaggtttgcccctctttacgcagtggaagccaaaagaatacagaaactagagcataccattaacaactacatacagttcaagagcaaacaccgtattgaaccagtatgtttgctagtacatggcagccccggaacaggtaaatctgtagcaaccaacctgattgctagagccatagctgaaagagaaaacacgtccacgtactcgctacccccggatccatcacacttcgacggatacaaacaacagggagtggtgattatggacgacctgaatcaaaacccagatggtgcggacatgaagctgttctgtcagatggtatcaacagtggagtttataccacccatggcatccctggaggagaaaggaatcctgtttacttcaaattacgttctagcatccacgaactcaagcagaatttccccccccactgtggcacacagtgatgcattagccaggcgctttgcgttcgacatggacattcaggtcatgaatgagtattctagagatgggaaattgaacatggccatggctactgaaatgtgtaagaactgtcaccaaccagcaaactttaagagatgctgtcctttagtgtgtggtaaggcaattcaattaatggacaaatcttccagagttagatacagtattgaccagatcactacaatgattatcaatgagagaaacagaagatccaacattggcaattgtatggaggctttgttccaaggaccactccagtataaagacttgaagattgacatcaagacgagtccccctcctgaatgtatcaatgacttgctccaagcagttgactcccaggaggtgagagattactgtgagaagaagggttggatagtcaacatcaccagccaggttcaaacagaaaggaacatcaacagggcaatgacaattctacaagcggtgacaaccttcgccgcagtggctggagttgtctatgtcatgtataaactgtttgctggacaccagggagcatacactggtttaccaaacaaaaaacccaacgtgcccaccattaggacagcaaaggtacaagggccagggttcgattacgcagtggctatggctaaaagaaacattgttacagcaactactagcaagggagagttcactatgttaggagtccacgacaacgtggctattttaccaacccacgcttcacctggtgaaagcattgtgatcgatggcaaagaagtggagatcttggatgccaaagcgctcgaagatcaagcaggaaccaatcttgaaatcactataatcactctaaagagaaatgaaaagttcagagacattagaccacatatacctactcaaatcactgagacaaatgatggagtcttgatcgtgaacactagcaagtaccccaatatgtatgttcctgtcggtgctgtgactgaacagggatatctaaatctcggtgggcgccaaactgctcgtactctaatgtacaactttccaaccagagcaggacagtgtggtggagtcatcacatgtactgggaaagtcatcgggatgcatgttggtgggaacggttcacacgggtttgcagcggccctgaagcgatcatacttcactcagagtcaaggtgaaatccagtggatgagaccttcgaaggaagtgggatatccaatcataaatgccccgtccaaaaccaagcttgaacccagtgctttccactatgtgtttgaaggggtgaaggaaccagcagtcctcactaaaaacgatcccaggcttaagacaaactttgaggaggcaattttctccaagtacgtgggtaacaaaattactgaagtggatgagcacatgaaagaggcagtagaccactatgctggccagctcatgtcactagacatcaacacagaacaaatgtgcttggaggatgccatgtatggcactgatggtctagaagcacttgatttgtccaccagtgctggctacccttatgtagcaatgggaaagaagaagagagatatcttgaacaaacaaaccagagacactaaggaaatgcaaaaactgctcgacacatatggaatcaacctcccactggtgacttatgtaaaggatgaacttagatccaaaacaaaggttgagcaggggaaatccagattaattgaagcttctagtttgaatgactcagtggcaatgagaatggcttttgggaacctatatgctgcttttcacaaaaacccaggagtgataacaggttcagcagtagggtgcgatccagatttgttttggagcaaaattccggtattgatggaagagaagctgtttgcctttgactacacagggtatgatgcatctctcagccctgcttggttcgaggcactaaagatggtgcttgagaaaatcggattcggagacagagttgactacatcgactacctaaaccactcacaccacctgtacaagaataaaacatactgtgtcaagggcggtatgccatctggttgctcaggcacttcaatttttaactcaatgattaacaacttgattatcaggacactcttactgaaaacctacaagggcatagatttagaccacctaaaaatgattgcctatggtgatgatgtaattgcttcctacccccatgaagttgacgctagtctcctagcccaatcaggaaaagactatggactaactatgactccagctgacaaatcagctatatttgaaacagtcacatgggagaatgtaacattcttgaagagattcttcagggcagacgagaaatacccatttcttattcatccagtaatgccaatgaaggaaattcatgaatcaattagatggacaaaagatcctaggaacactcaggatcacgttcgctctctgtgcctattagcttggcacaatggcgaagaagaatataacaaattcctagctaaaatcaggagtgtgccaattggaagagctttattgctcccagagtactcaacattgtaccgccgttggcttgactcattttag

SEQ ID NO: 2 - DNA, 6630 bp, Artificial Sequence
  optimized STR
atgggagctcaggtatcttctcaaaaagttggggcccatgagaactctaacagggcgtacggggggtcgaccataaactacaccaccataaattattatagggactctgcctcgaacgcggcctcgaaacaagacttctcgcaagacccgtccaagttcaccgagccgataaaggacgtcctcataaaaaccgcacccatgctcaactcgcccaacatagaggcctgcgggtactcggacagggtcctccaactaaccctcggtaactccaccataaccacccaagaggcggccaactctgtcgtcgcctacgggcgttggccggagtacctccgcgactcggaggcgaaccccgttgaccaaccgaccgagcccgacgtcgccgcctgccgcttctacacgctcgacaccgtttcgtggacgaaagagtcgcgtgggtggtggtggaagttgccggacgccctcagggacatgggtttattcgggcaaaacatgtactaccactacctcgggcgctccgggtacaccgttcacgtccaatgcaacgcgtccaaattccaccaaggggccctcggagtcttcgcggtccccgagatgtgcctcgcgggcgactcgaacaccaccaccatgcacacctcgtaccaaaacgcgaacccgggggagaaaggtgggaccttcacggggacgttcaccccggacaataaccaaacctctccggcgcgtcgcttctgcccggttgactacttacttggtaacgggacgctacttgggaacgcgttcgttttcccgcaccaaataataaacctccgtaccaacaactgcgccaccctcgtcttaccgtacgttaactccttatcgatagactcgatggtcaagcacaacaactggggtatagccatactacccttggcgcccctaaacttcgcctcggagtcctcccccgagatacccataaccttgaccatagcgccgatgtgctgcgagttcaacggtctaaggaacattaccctcccccgtctacaagggctcccggtcatgaacacaccggggtcgaaccaatacctaaccgccgacaacttccaatctccgtgcgcgctcccggagttcgacgttacccccccgatagacataccgggggaggtcaagaacatgatggagttggccgagatagacaccatgataccgttcgacctatcggccaccaaaaagaacaccatggagatgtaccgcgtccgtctatcggacaaaccccataccgacgacccgatattatgcctctctttatcgcccgcctctgacccgcgcttgtctcacaccatgctaggtgagatactcaactactacacccactgggccggttccctcaagttcacgttcctcttctgtggttttatgatggccaccgggaaactcttggtttcttacgcgccgccgggtgcggacccccccaagaagcgtaaggaggcgatgttgggtacccatgttatatgggacataggtctccaatcctcttgtaccatggtcgttccctggatatcgaacaccacgtaccgtcaaaccatagacgactcgttcaccgaggggggttacatatcggtcttctaccaaaccaggatagtcgtcccgctatcgaccccgagagagatggacatactagggttcgtttctgcgtgcaacgacttctcggttcgtttgatgcgtgacaccacccatatagagcaaaaagcgctcgcccaagggctagggcaaatgctagagtcgatgatagacaacaccgtccgtgagacggttggggcggccacctcgagggacgccttacccaacaccgaggcgtcgggtcccacccactccaaggagataccggccttaaccgccgttgagaccggggcgaccaaccccctcgtcccgtcggacaccgttcaaaccaggcacgtcgtccaacaccgctctcgctctgagtcgtcgatagagtcgttcttcgcgcgtggggcctgcgttactataatgaccgttgacaaccctgcctccaccaccaacaaggacaagctcttcgccgtttggaagataacctacaaagacaccgtccaactacgtcgcaaattggagttcttcacctactcgaggttcgacatggagttaaccttcgttgtcaccgccaacttcaccgagaccaacaacgggcacgcgctaaaccaagtttaccaaataatgtacgtcccccccggggcccccgttccggagaaatgggacgactacacctggcaaacctcttctaacccctctatattctacacctacggtaccgcccccgcgcgtatatcggtcccgtacgtcgggatatcgaacgcgtactctcacttctacgacgggttctccaaagtccccctcaaggaccaatcggccgccctcggggactccttatacggggccgcctcgctcaacgacttcgggatattggccgtcagggtcgtcaacgaccacaacccgaccaaggtcacctccaaaataagggtttacctcaaaccgaaacacataagggtctggtgcccgcgtccaccgcgcgccgttgcgtactacgggccgggtgttgactacaaggacgggacgctaaccccgttatccaccaaggacctcaccacctacggtttcggtcaccaaaacaaagcggtttacaccgccgggtacaaaatatgcaactaccatttggcgacccaagacgacttgcaaaacgccgttaacgtcatgtggtcgagggacttactagtcaccgagtctagggcgcaagggaccgactctatagcccgctgcaactgcaacgccggggtttactactgcgagtcgaggcgcaaatactaccccgtctccttcgtcgggcccacgttccaatacatggaggccaacaactactaccccgcccgctaccaatcccacatgttaatagggcacggtttcgcctcgcccggggactgcggggggatattaaggtgccaccacggggttatagggataataaccgccgggggagaggggttggtcgccttctccgacataagggacttgtacgcgtacgaggaggaggcgatggagcaagggataaccaactacatagagtctctaggggcggccttcggttcgggtttcacccaacaaataagtgacaaaataaccgagttgacaaacatggttacctcgaccataaccgagaagctcctaaagaacttgataaagataatatcctctctcgtcataataacccgcaattacgaggacaccaccaccgttttagccaccctcgcgctactagggtgcgacgcctctccctggcaatggctaaggaagaaagcctgcgacgtcctcgagataccgtacgtcattaagcaaggggactcgtggttgaagaagttcaccgaggcctgcaacgccgccaagggtctcgagtgggtttctaacaaaatatctaaattcatagactggttaaaggagaaaataataccccaagccagggacaagttggagttcgtcaccaaactaaggcaactcgagatgctcgagaaccaaatatctaccatacaccaatcttgcccgtcgcaagagcaccaagagatactcttcaacaacgtcaggtggctatccatacaatcgaagcgcttcgcgccgctatacgccgtggaggcgaaaaggatacaaaaactcgagcatactattaacaactacatacagttcaagagcaaacaccgtattgaaccagtatgtttgctagtacacgggtcgccgggtaccggtaaatcggtcgccaccaacctcatagccagggcgatagccgagagggagaacacgtccacgtactcgctcccgccggacccctctcacttcgacggttacaaacaacaaggtgttgttataatggacgacctcaaccaaaaccccgacggggcggacatgaagctcttctgtcaaatggtctctaccgttgagttcatacccccgatggcctccctcgaggagaaaggtatactcttcacctctaactacgtcctcgcctccaccaactcttcgaggatatccccgccgaccgttgcccactcggacgccctagcgcgccgtttcgcgttcgacatggacatacaagtcatgaacgagtactcgagggacgggaaattgaacatggcgatggccaccgagatgtgtaagaactgtcaccaacccgccaacttcaagaggtgctgcccgctagtttgcgggaaggccatacaactaatggacaaatcgtccagggtcaggtactcgatagaccaaataaccaccatgataataaacgagaggaacaggaggtccaacatagggaactgtatggaggccttgttccaaggtcccttacaatacaaagacttgaagatagacataaagacgtcgccgccgccggagtgcataaacgacttgttacaagccgtcgactcccaagaggttagggactactgtgagaagaaggggtggatagtcaacataacctcgcaagtccaaaccgagcgcaacataaaccgcgccatgaccatactccaagcggttaccaccttcgcggccgttgccggtgtcgtctacgtcatgtacaaactcttcgccggtcaccaaggtgcctacaccgggctacccaacaaaaaaccgaacgttccgaccataagaaccgccaaggtccaagggcccgggttcgactacgccgttgccatggccaaaaggaacatagtcaccgccaccacctcgaagggtgagttcaccatgctaggtgtccacgacaacgttgccatactacccacccacgcctctccgggggagtcgatagttatagacgggaaagaggttgagatattggacgcgaaagcgttagaggaccaagccggtaccaacctagagataaccataataaccctcaagaggaacgagaagttcagggacataaggccccacataccgacccaaataaccgagaccaacgacggagtcttgatcgtgaacactagcaagtaccccaatatgtatgttcctgtcggtgctgtgactgaacagggatatctaaatctcggtgggcgccaaaccgcccgtaccctcatgtacaacttccccaccagggccggtcaatgcgggggtgtcataacctgcaccgggaaagtcatcgggatgcatgttggtgggaacggttcacacgggtttgcagcggccctgaagcgatcatacttcacccaatcgcaaggggagatacaatggatgaggccgtcgaaggaggttggttaccccataataaacgcgccgtccaaaaccaagctagagccgtcggccttccactacgttttcgagggggttaaggagcccgccgtcttaaccaaaaacgacccgcgcctaaagaccgatttcgaggaggccatattctccaagtacgttgggaacaaaataaccgaggttgacgagtatatgaaagaggccgtcgaccactacgccgggcaattaatgtctctcgacataaacaccgagcaaatgtgcttggaggacgcgatgtacgggaccgacgggctcgaggccctagacttgtccacctcggccgggtatccgtacgtcgccatgggtaagaagaagagggatatattgaacaaacaaaccagggacaccaaggagatgcaaaaactcttagacacctacggtataaacttacccctcgttacctacgtcaaggacgagctaaggtccaaaaccaaggtcgagcaagggaaatccaggctaatagaggcctcgtcgttgaacgactctgttgccatgaggatggccttcgggaacctctacgccgccttccacaaaaaccccggtgttataaccgggtctgccgtggggtgcgaccccgacttgttctggtcgaaaataccggtcttgatggaggagaagctcttcgccttcgactacaccgggtacgacgcctcgttatcgccggcctggttcgaggccctcaagatggttctagagaaaataggtttcggtgacagggtcgactacatagactacctcaaccactctcaccacctctacaagaacaaaacctactgcgtcaagggggggatgccctcgggatgctctgggacctctatattcaactctatgataaacaacttgataatacgcaccttactactcaaaacctacaaggggatagacctagaccacctcaaaatgatagcgtacggggacgacgtcatagcctcctacccccatgaagttgacgctagtctcctagcccaatcaggaaaagactatggactaactatgactccagctgacaaatcagctacatttgagaccgtcacctgggagaacgtcaccttcttgaagaggttcttccgcgccgacgagaaataccccttcctaatacaccccgtcatgcccatgaaggagatacacgagtctataaggtggaccaaagacccgcgcaacactcaggatcacgttcgctctctgtgccttttagcttggcacaatggcgaagaagaatataacaaattcctagctaaaatcaggagtgtgccaattggaagagctttattgctcccagagtactcaacattgtaccgccgttggcttgactcattttag